European Patent Application EP 4 365 188 A1, published May 8, 2024. Title: Method for preparing micrococcin-based carboxylic acid compound and micrococcin-based carboxylic acid compound prepared therefrom. Applicant: A&J SCIENCE CO.,LTD. The sequence listing filed with the application follows.

SEQUENCE LISTING (3 sequences)

SEQ ID NO: 1 - DNA, 18647 bp, Artificial Sequence
  Plasmid 1 - Example 2
tcgcgcgtttcggtgatgacggtgaaaacctctgacacatgcagctcccggagacggtcacagcttgtctgtaagcggatgccgggagcagacaagcccgtcagggcgcgtcagcgggtgttggcgggtgtcggggctggcttaactatgcggcatcagagcagattgtactgagagtgcaccatatgtttgcaaaacgattcaaaacctctttactgccgttattcgctggatttttattgctgtttcatttggttctggcaggaccggcggctgcgagtgctgaaacggcgaacaaatcgaatgagcttacagcaccgtcgatcaaaagcggaaccattcttcatgcatggaattggtcgttcaatacgttaaaacacaatatgaaggatattcatgatgcaggatatacagccattcagacatctccgattaaccaagtaaaggaagggaatcaaggagataaaagcatgtcgaactggtactggctgtatcagccgacatcgtatcaaattggcaaccgttacttaggtactgaacaagaatttaaagaaatgtgtgcagccgctgaagaatatggcataaaggtcattgttgacgcggtcatcaatcataccaccagtgattatgccgcgatttccaatgaggttaagagtattccaaactggacacatggaaacacacaaattaaaaactggtctgatcgatgggatgtcacgcagaattcattgctcgggctgtatgactggaatacacaaaatacacaagtacagtcctatctgaaacggttcttagacagggcattgaatgacggggcagacggttttcgatttgatgccgccaaacatatagagcttccagatgatggcagttacggcagtcaattttggccgaatatcacaaatacatctgcagagttccaatacggagaaatcctgcaggatagtgcctccagagatgctgcatatgcgaattatatggatgtgacagcgtctaactatgggcattccataaggtccgctttaaagaatcgtaatctgggcgtgtcgaatatctcccactatgcatctgatgtgtctgcggacaagctagtgacatgggtagagtcgcatgatacggaattcgagctcggtaccgaactcctttttcatatgagaaggtgccatgtcactattgcttcagaaatactcctagaataaaaaaactcatctttaaagatgagctgtccattccataaaaaattacattgtaatcatgtccagaaaatgatcaatcacaatggaggacattcctaatgccggtgcattctgtcctaaggaagatggcaataattcatagctattgcctaattgggaataaacccttgatgatacttcacttctcattgaatttaaaaccataggatgcgattcaattatgctatttcttaaaattacggcttgtgggttgaaagtatttagaatattggtaaggcctattcctaaatagaatccaaaattttgtaatgcatttaaggttccgatatcattcagatgggcgaggtttatgatatcttgataggacagttttttctctttggtctgaagagattttaataaagccttctctgaagcatacaattcccagcatcctcggtttccgcaactgcatttaggaccattaaagtctattgtcatatgtcccatttctccagagaagccgcttactcctctatataaatgattgttgataataacaccgatccctattcctgtgctgatacttacgtaaataatgttatcgtgattttttgcagctccaaatactttttctccatatgcgccagcatttgcctcattttcaataaaaacaggcacattgtacttctcttgtatcgaagattttaagtcaatatctctccagttggagttcggagtgaaaacaattttttgatctttatcaatgagtccaggcacgcaaatacctataccaataagcccgtacggagattggggcatttgcgtaataaagtgatgaatcatatcaatcaaaatgtctttcgttatttctggagaattggattccaaatggcggtattgatcaagaacgattgttccttcaaggtctgttaaaatgccattaatataatccacaccaacatctattccaacggagtatcctgcctttttattaaaaacaagcatgacaggtcttcttccgccacttgattgtccttgacctatttcaaataccatactttctttcattaacgtgtttacctgtgatgagacagttgatttatttaatccagtcatttcagataattttgctcttgaaataggtgaatttttaaggatttcttttaataataacttttgatttacttttttgacaaaggtttgatcagcgatatccacttcatccactccatttgtttaatctttaaattaagtatcaacatagtacatagcgaatcttccctttattatatctaatgtgttcataaaaaactaaaaaaaatattgaaaatactgacgaggttatataagatgaaaataagttagtttgtttaaacaacaaactaataggtgatgtacttactatatgaaataaaatgcatctgtatttgaatgaatttatttttaagggggaaatcacatggctcaatctcattccagttcaatcaactattttggaagcgcaaacaaagtggtttactaaggtacccgggctagctttaagaaggagatatacatatgagtgaaattaaaaaagcattaaatacgcttgaaattgaagattttgatgcaattgaaatggttgatgttgatgctatgccagaaaacgaagcgcttgaaattatgggagcgtcatgtacgacatgcgtatgtacatgcagttgttgtacaacttaatctagctttaagaaggagatatacatatgagtgaaattaaaaaagcattaaatacgcttgaaattgaagattttgatgcaattgaaatggttgatgttgatgctatgccagaaaacgaagcgcttgaaattatgggagcgtcatgtacgacatgcgtatgtacatgcagttgttgtacaacttaatctagctttaagaaggagatatacatatgagtgaaattaaaaaagcattaaatacgcttgaaattgaagattttgatgcaattgaaatggttgatgttgatgctatgccagaaaacgaagcgcttgaaattatgggagcgtcatgtacgacatgcgtatgtacatgcagttgttgtacaacttaatctagctttaagaaggagatatacatatgagtgaaattaaaaaagcattaaatacgcttgaaattgaagattttgatgcaattgaaatggttgatgttgatgctatgccagaaaacgaagcgcttgaaattatgggagcgtcatgtacgacatgcgtatgtacatgcagttgttgtacaacttaactcgagcaccaccaccaccaccactgacgtacgggcccaagcggtacccggggatccgtttgttccctttatagaaaggaatgatcaaatgttagaaataaaagaaaaacaatttattaaattaaaagaggacacattcttttttccttcagctgaagggatatactttaggaattctataggttattttacaatcaaaggtagaaatatttacccgttttttagtgaaatcagtaaatatttgaatggtaaatatactttgaaagatatagtgagtgagttaagcaaaacccaagaagaaaaatttttaaaattaattgccatattagagaagaatggttttgtaaaatataccgaaagggttattgatgaaaattattataaaaattatgaaaaagaaattgcatttatagattattatactaataatggcatcgaattatttaaaaaactctctaatttcaagatttgtttatatggtagcaataagttatctaatactattcaaaaaagcttagaaaacatagggatacaaaatattaaaagaggctctcgttttgattttgagggagacattgttatttattgcaataatgatgttaatgaaagggaaaatctactggaatgtatggacttttctcagaataaaatatttatttttgtaggtaataaagaatcattaggaattattagtcctattataaaaaatttagatgattggaaggaatttgaaaatatattagagattggtgcagataatattaaagaaaatacaacatttactagcaactctatattaagtagtatgctaagttttgaaattataaagtatgtaacaaattgtttgcaaagtgatttaattaatgcggcatacattttaaatactgatactttaaaagggaattttgttcaggtaaaaaaaaaaatagacttaaaacaagattttattgaaactttcaaacaatcaagcggaggcaacggtttgtatatcaataaaataggtagaggttctaggaaacaaattccgctctcgcaatgggaggttgaattggataaattaggtgacatgaatagtgaaaaaattaaggtcgttagctttggtgatacccaccaggaagcgaggtttaatacttattataaaaccatagaacatctaataatcaatggggaatttaacttagaggaatcatatagctttaagaatcttgatacaatcactttagctattgatgaacaatttaaaagaaaattaacaatttcatgcgacatagataaagaacttgcaatcagaaaagcaatattaaaagcaattttaaagagggaaattaatgtaattgataattatcaagagctttccccattaaaaataagtgattatatagataataaaaatatacaatactattgtaaactgattaacattttaaaagcgaaaatagaattgcgttttaagaaattagtagagggtttgtttttggtagtagttagtgacaatagttataggggagttagtataggatttaatttaaatacagcattagaaaatgctcttaggcaatttattaataatttacaaaatagtatctatacaataaatattgaagatgtaatatttaaaagaattaatgattgggatgatgaatgcattcgagagtttttgacagatgaaaaattagaagtttttatctgtagtatacaaaataatgttatttcagcagaaatttctatagttggagcaatattaatagaaagttaggtgaattgaaaaatgaataaggaagtccttataatcagggatgaaagctttggagaattttttgattctttttttttaaatgaaaataatcgaaaagtttgttttatagatagtaataaaaaagatttgaaatatttattaaaaaactttttagagaataaaaagtttagttatgtactaatctttccaaaggaatggaatcctatgatgtataggtcacttgatgcagtgttagaagactatgatgtaccgtggatctatataacacaattttttaataaaattttaataggtccttttagaaattctaagcaaaaaggttgtttagattgtttatattatagatggtttatgacaaaaaaggatcgtattaatttatttgaattgaagaaatgtttatcagaaggacataatgtaaaaatatctggagatttattgaatgcttcaatggttggattagcaattactttagcatttaaactaataaataatgaggtttcggaattttcgtatattattgacaaaaagacattgagattcaatggtcataattttttacctaatccacattgtcaagtatgtgggcacatggataatgacgagaaaagattaatagaacacaaattttttacagcacttaacgataatactcttaaagaaaagaaaggaaatcgttttttatcaaaagaatatttagaagataccctatctaaaaattttttagatgtagaaactggtatatttaataaacttttggacgattatgaaagtcctttcgcagtttcggtagcaaatcttcctttaaaggttggaaaggatgaggttggtgttggaagaacggataattatgctaatagtcacttaactgcaatattagaaggaatagagagatattgcggaatggaaccaagggggaatagaactaacgtttttggtagttataatgagctaatggaaaatgctctcaatccatctgttttaggattacacgcggaagaacagtatcaattaaaaagatttccttttaataaatataatccagataaaaaaatgaaatgggtctgggggtattcttttaataagaataaggcgatattagtccctgaaacttatgcctattatggtacgaattatagagatggcgttcaaaatagttttgtttatgaaatctcgaatggatgtgctttaggaggacatttattggaagctacattgcaaggaatttatgaagtagtggaaagagatgcttttcttatatcttggtatactaaattaccattaaaacgtataagaaaagaatctattaaggatcagacgattcaattattattaacgagatttgaatatcaaactgattatgatattcatctgtataatatgactttagagaataaaataccaactattttagctattgcaaaaaatagaggtgcttttggcatgaatattttatgtgctgcaggttgtcatttagatataaataaagcaattgaaagttcattacatgagttatgtggaatcttagaggcaatcaaaagtaaatttgaaaataggaaaagtgaattatacgaaatggcaaagaattattcacttgtacggacgatggaagatcattcattattatttggattgaaagaacttgaaaaagagtttgattttctattaaagagcccgattgaaattgatttaagtgaggtagaacctttaaaatatagcaacaatatacatacagatttattgaatgtaattgattattttaaaaaaataaatttagatatcatcgtagtcgatcaaaccgcggaagatataaaatttaacaacttgtattgtgtaaaagttattattccaggaatgttacctatgacatttggacatgatatgagaagaatacataatttaccaaggatattccgtgttccaagggaattaggacataaaattaagaatgaaaatgaaattaagaacaatcaggtaactcctcatcctttcccataacattttttatgaaagatggtgatataacatgaaaccaataaactatgtaccacattttttatgtagaatatctggtgaagaaataaactctatttcagaaattgagtttattaaaaccttggaatgtttagaattatccgaaggaattttaaggaaaataaattctttatcagcagacttaacgaaagatttacatgattgtatttctttatataaagaacaatctatttcacgtgtattaataaatcttaaaagagatatttttaatatgaggtttaatcgagttcaaaagtataaactagaaaatatctcaggttttaaccacgataaattaaatttatggttaaatttagctcaagaatatcaaagcacgctacatctgatgagagaaacttttaaaatggaaatacaggaaaaaagagggaaattaaagcagttatttagtaatagtgaatatataaaagccattcaagtctcaaatactcaactttatgaaaatctcctagaatacttacaagataatcaaagtcatcctccaaaaaagatgaggaatattgaacagtctctaattaattacctaagtcgtatgatatttaagccaactcccttcagttcatttacaggattaaattacggtttttttagtcaggaagattcaagttttgaaataaatactaaggaaagcaaaggtcacactcgaataaacatggtttatttaaaaaaaattgaaagaatgttattaaatcgaatatctataaaaaataaatgttatgtttcgttaaatcaaacgataaacgaagaggaaaattatatgttttttcgaagaggtaaagatgggactagtcaagcttttactggtgaagcttttataaagataaaaaagagcgagctcttaaaggagttaattcaatattttgaaggaatatcttcaatgaatatagttgaggttgtatcatttctttccgaaaaaacaaattatgaaactgaagctttatataattacttatttaagttagagaaaatgggagtgttagattttagcttaggtgtgtccgaacaatcggacaattacacgaaagatttgatagaaaacttattggggattaaagattcattagttgaaaaatcggtctcacaccttgtagaaatagaaaaaattcaggcgattttctctgaatccaattaccaaaaacgttatgtacttttaaaaaatttacaagaacatataaagaagatttatagtttatttgatttaaaattagagtctaatgatttgacctctctattattcgaggatgttagttataaaaatactaagattatattaaatgaaaatcaatggaaaacgcatcttgatgattttaatttaattaagaatttaatgccactttttgatgataatatccttgaaaaattaagtatgaatataatttttaaggatatatatggtaacaagggggcaatagatttattagaattctatagagagtttaataaatatgataaaaatttattatggaagaaaattagaaaaaatgatacatatctttatttaaaaaaattgagaacagagttttatgattatctagaaacacaaattaatatggggttagacactatctttttaaataaaagttggttaaagaaatttattaacaagttccctgatttattgaagagtaaggaaaattattctttctattttcaaatagcctatgataatcaagataatagaattttagttttaaataagatagggccaggattaggtaagcacttttcaagatatggtaatttatttttaaatagcgaatacaaggaaaataatagatttattaattctcttatagaacagtataaaaaatatgatcaaaatgggggggttttaacagatttaaatgcagtgttaggtctaaatcttaatatgcatcctaatcttttaaattatgaaattacttatccaggatgcaatcctagtaaaggaattaatcaagtagcattaaaggatattgaagtattgtatgattctaattctgaccaactaaaattatattctaaacaatatagacagaatgttaaattacttccattgggatttttgtttccagcattgtccccatctttatataagtttttatgtggattttcggaatcaaatgggatagagtattctttttggaacaagttcttaaatgaacacaataataatttttcacttttacctagaattatgttaggatcagtagctttggatagaagaacatggaaaattaatgcgaaggaaatacaaaaggaattttctaaagatacatttgaaacttttattaacttccataagtgggtgaaagaaaatcaactaccggaagatatatttttaagggttgcaaacacaatggacgcttttagtgagaatgaattattaaatcaagatttaggaagttggattgcagaaattaaacaaactaaacatcgtaaacctcaatatgttaattttaataattactttcatatcgatgccttaagaaagattattaaagatgttaataatacagtaacaattcaagaagtttatcctcatccagatgatgtgtattatcaaaaaaatagtaaaaaatgtgtagaatttttagttgaggttttttaataaaggaatgattatatgaacgagaataattttatatggaaggcttatcatattttttatcatcaaaatcaagattttctaattacaaattgtatcaaaccaattttagatgaattgataaaaaagaaattaattagtaaatttttttttataagatattgggaaggcggacctcatattagagtgcgactttattgtacattaaataaatctcaagaagttgattataaatttaatgattttgtttctaaattcttgaaaacatatccttcttcatcaacattagatagaaacatgataaagaatcaattagcaaaattagctagtcttgaagagggtactgagtcaacatgtgttcgagagaataatcatattattcatctagaatataatccagagtataaacgatatggaggagaaaatggaatagagattgcggaagaacatttttaccattcaagtataatgtgtttgaagttaatacaagaaattaataaaaagacaaatcgtttgcgcatatctattgaaattatactatcttatttaaaagctatgaatatgaacttacaagagagtattaagtttttagaaggctattatctaatatggaaaagatatgtatacagcaataccaataacgttgaagaattcttcgctaacaaatatattaagcaaaaaaaagtaatagacaaaattgtagtaaactatttcaattctaataataataaaggtatgttaggagaaaaatggagtaatcatttgaatttaactgtacagaatttagaaaatgattgggatcggggagaattaataatagataaagatgttttagcatatataaatatccctcaaaagattgcttttatagttacaagttatgttcatatgacaaacaataggcttggtatcatgccgcaagaagaagcctatttaagctatatgcttttatgtagtttgaaatcattgtataagagtagaaagggatgacttaaatggagcagtatcataaaattgtattaactggaagtaatgctgagactatgttaataaaaaatatagagcctgtagcagttaagtttataaataactataagggttttttctatgtttttaaatatagtaaagattttccaattatcgatgtttatatcaacaacaaaattgttacagaaaatcaattaaataaaattttacagaattctggggctaaatataaaatttataaaaattcaatatttaatgagacacaagggaattttgggatgttaggtgataaatatctggcagaattttttaaaaagacaaatgaaattagccttaatatactaaatcaaaattttgagagttacaataaaaaaatagaatttgcgctagagataatgttaatttcagcgcactataattatgattcaataaaaaaaggctacttatcctatgcatctcatgtaaatggattttttactagatggaaagatccaaataaaattagagatatatttcataagaactacttaaataacaaagagtacctagaatcgaaagtttcagaaataatagataataacaacagaagtagcttgagcgaattatcggatattattacagaaatgaagaaagagatgactactgatattgagaaggggaacctgcatgtatttaatattgaattactacaaaaaccaggagaaagagattttctagaaaaaagtcagtttcataagacgatattaaataatccagatttctctaattttatgaataaagatataaactttttaggttcacgcctaataactgtatttacgtacttattaatacgaaatttagggattcaaaataaagatagatatctactttgctactatatctataaaattattgaagaaaaatataatatagatactttggaattaataagggattttggtaaagggagggataataatgttgaagacttacaaagatattgaagattttttatataatttgcaatattcgcctgctaaagcttcagatttcaatttagatttaagtaattatgatagacccttgccttttaaaatttataggaatagagaatcgatagatttagacgataactttccgatttgtattaatgatttagatggtattgattattcaaatttcgaaattattagttatttattgtggtatacctatggttttaccagctacaattggttaacaaaaccaacattaaatggtcagaatacatccttaagtttttttagaagaagtgtagcctcaggtggcggcttatatcctggggaaatttacttatatgtggagagtattaaaggtatcaagtcaggattatattattttgatgttaggggaccgagattaattttactaagggaaggaaattttcaagaatttatcaaaaaatctttgcaatataatcaagatagaaatgtttatatttttataacatcattttattggaaaaacttctttaaatatttaaatttctcgtatcgtttacaaggcttagatatcggtgctattgtaagccaagctcacctaatttcaaagaaattaggtcttaattcggagattaggtatcactttgatgataaaaaaattaatgattttttaggaatcaacgctgaggaagaaagcagctacgtagttttgcctatagatatggataataattcatataaaagtgaaaataaggttcccgcttttgagtactttaaaaacgatacaacattcaattatattgaacatttaaatgttggccccaaaaatgtatgtcaggatatttataaaatcaatagtaatattatcaatagtggcttaattaaagttaaaaaaaatgaaatagcatcttttaaagaggaggcaaatgttgttcataaagaaaaatatgattatgacattttgaaggcttctgtaagtcgtatatcaccaggagagaactttttgtctgattttttgaatattcagcatgttcacaaagttctagatgttggaatgcaggaacaatttaaaaatgatatttttagcgataattatagtgttctaaaggatgttgaaatttacttttatgccaataagattgaaggtttaccaaaaggctactattactataatccaagtaataaaagtttcgttttgaaacataaaggtgatttttctagtgtttttcaggagaatcttacacgaaaaaattttaatttagtagaaatgcctttaattgtgcacttagtattaaacatgaaaaaatttatagaaaatatgaaatttagaggctatagagtcatgcaaatggaggcagggagaattatgcatcaaatacaattgaatgctgcaggtttgaacctagggagccatccaatgttaggttatagggctgataatttggaggagttttttggtattcaaaataatataactgtccagatgtctattggtaaatatagacctttattgaggctaaccaataatttattgaataaaactaaaggagaacaattttatgtatgacggaaaacgggtgaatccatatgaactctatcaaacaatttaattttaaaaataaaaatatttttattactggagctaccagtgatatagctatctgtatagcagaatccttctctggatttggcgggaatttaattttatctgatactgataaacaattaccaaaattagaacatgttaaacaaaaaatgattgaaaaatttaggaataatgttcaaattgtaactattgatttatataaggttaatgatatacaaaatgcaattgaaaaattagataaaccaattgatatattgatcaattgtgctggaaataattactttgttccagctctggaggttagtgaagagaattggcaaaaaattatagatgtaaatttgaaaggaactttttttcttagtcagtcaatagcaaaaaaaatgattagtgacggcataaaggggaaaattgtaaatattggatcgcaacatggggtagttgccaatggtctaagagccccctattgtattagtaagtttggattaataggtttgacaaaagttttagcgctagagtggtctacttttaatatattggttaattgtgtttcaccaacgtatgtaaaaacttctaaaagtaaggatttcttggagcatgaagatgttaaaaaagcatatttatataaaatccctttgaaaaaatatgctttaccccacgatatatcatatgcagtattgtttttaagtagcgatcaaaatcagataattacaggggaaaatattttagttaatggtggttatacattacactagatctcaccaccaccaccaccactgacgtacgggcccaagcttgcacccattagttcaacaaacgaaaattggataaagtgggatatttttaaaatatatatttatgttacagtaatattgacttttaaaaaaggattgattctaatgaagaaagcagacaagtaagcctcctaaattcactttagataaaaatttaggaggcatatcaaatgaactttaataaaattgatttagacaattggaagagaaaagagatatttaatcattatttgaaccaacaaacgacttttagtataaccacagaaattgatattagtgttttataccgaaacataaaacaagaaggatataaattttaccctgcatttattttcttagtgacaagggtgataaactcaaatacagcttttagaactggttacaatagcgacggagagttaggttattgggataagttagagccactttatacaatttttgatggtgtatctaaaacattctctggtatttggactcctgtaaagaatgacttcaaagagttttatgatttatacctttctgatgtagagaaatataatggttcggggaaattgtttcccaaaacacctatacctgaaaatgctttttctctttctattattccatggacttcatttactgggtttaacttaaatatcaataataatagtaattaccttctacccattattacagcaggaaaattcattaataaaggtaattcaatatatttaccgctatctttacaggtacatcattctgtttgtgatggttatcatgcaggattgtttatgaactctattcaggaattgtcagataggcctaatgactggcttttataatatgagataatgccgactgtactttttacagtcggttttctaatgtcactaacctgccccgttagttgaagaaggtttttatattacagctccagatcctctacgccggacgcatcgtggccggcatcaccggcgccacaggtgcggttgctggcgcctatatcgccgacatcaccgatggggaagatcgggctcgccacttcgggctcatgagcgcttgtttcggcgtgggtatggtggcaggccccgtggccgggggactgttgggcgccatctccttgcatgcaccattccttgcggcggcggtgctcaacggcctcaacctactactgggctgcttcctaatgcaggagtcgcataagggagagcgtcgacatggatgagcgatgatgatatccgtttaggctgggcggtgatagcttctcgttcaggcagtacgcctcttttcttttccagacctgagggaggcggaaatggtgtgaggttcccggggaaaagccaaataggcgatcgcgggagtgctttatttgaagatcaggctatcactgcggtcaatagatttcacaatgtgatggctggacagcctgaggaactctcgaacccgaatggaaacaaccagatatttatgaatcagcgcggctcacatggcgttgtgctggcaaatgcaggttcatcctctgtctctatcaatacggcaacaaaattgcctgatggcaggtatgacaataaagctggagcgggttcatttcaagtgaacgatggtaaactgacaggcacgatcaatgccaggtctgtagctgtgctttatcctgatgatattgcaaaagcgcctcatgttttccttgagaattacaaaacaggtgtaacacattctttcaatgatcaactgacgattaccttgcgtgcagatgcgaatacaacaaaagccgtttatcaaatcaataatggaccagacgacaggcgtttaaggatggagatcaattcacaatcggaaaaggagatccaatttggcaaaacatacaccatcatgttaaaaggaacgaacagtgatggtgtaacgaggaccgagaaatacagttttgttaaaagagatccagcgtcggccaaaaccatcggctatcaaaatccgaatcattggagccaggtaaatgcttatatctataaacatgatgggagccgagtaattgaattgaccggatcttggcctggaaaaccaatgactaaaaatgcagacggaatttacacgctgacgctgcctgcggacacggatacaaccaacgcaaaagtgatttttaataatggcagcgcccaagtgcccggtcagaatcagcctggctttgattacgtgctaaatggtttatataatgactcgggcttaagcggttctcttccccattgatagcttggcgtaatcatggtcatagctgtttcctgtgtgaaattgttatccgctcacaattccacacaacatacgagccggaagcataaagtgtaaagcctggggtgcctaatgagtgagctaactcacattaattgcgttgcgctcactgcccgctttccagtcgggaaacctgtcgtgccagctgcattaatgaatcggccaacgcgcggggagaggcggtttgcgtattgggcgctcttccgcttcctcgctcactgactcgctgcgctcggtcgttcggctgcggcgagcggtatcagctcactcaaaggcggtaatacggttatccacagaatcaggggataacgcaggaaagaacatgtgagcaaaaggccagcaaaaggccaggaaccgtaaaaaggccgcgttgctggcgtttttccataggctccgcccccctgacgagcatcacaaaaatcgacgctcaagtcagaggtggcgaaacccgacaggactataaagataccaggcgtttccccctggaagctccctcgtgcgctctcctgttccgaccctgccgcttaccggatacctgtccgcctttctcccttcgggaagcgtggcgctttctcatagctcacgctgtaggtatctcagttcggtgtaggtcgttcgctccaagctgggctgtgtgcacgaaccccccgttcagcccgaccgctgcgccttatccggtaactatcgtcttgagtccaacccggtaagacacgacttatcgccactggcagcagccactggtaacaggattagcagagcgaggtatgtaggcggtgctacagagttcttgaagtggtggcctaactacggctacactagaagaacagtatttggtatctgcgctctgctgaagccagttaccttcggaaaaagagttggtagctcttgatccggcaaacaaaccaccgctggtagcggtggtttttttgtttgcaagcagcagattacgcgcagaaaaaaaggatctcaagaagatcctttgatcttttctacggggtctgacgctcagtggaacgaaaactcacgttaagggattttggtcatgagattatcaaaaaggatcttcacctagatccttttaaattaaaaatgaagttttaaatcaatctaaagtatatatgagtaaacttggtctgacagttaccaatgcttaatcagtgaggcacctatctcagcgatctgtctatttcgttcatccatagttgcctgactccccgtcgtgtagataactacgatacgggagggcttaccatctggccccagtgctgcaatgataccgcgagacccacgctcaccggctccagatttatcagcaataaaccagccagccggaagggccgagcgcagaagtggtcctgcaactttatccgcctccatccagtctattaattgttgccgggaagctagagtaagtagttcgccagttaatagtttgcgcaacgttgttgccattgctacaggcatcgtggtgtcacgctcgtcgtttggtatggcttcattcagctccggttcccaacgatcaaggcgagttacatgatcccccatgttgtgcaaaaaagcggttagctccttcggtcctccgatcgttgtcagaagtaagttggccgcagtgttatcactcatggttatggcagcactgcataattctcttactgtcatgccatccgtaagatgcttttctgtgactggtgagtactcaaccaagtcattctgagaatagtgtatgcggcgaccgagttgctcttgcccggcgtcaatacgggataataccgcgccacatagcagaactttaaaagtgctcatcattggaaaacgttcttcggggcgaaaactctcaaggatcttaccgctgttgagatccagttcgatgtaacccactcgtgcacccaactgatcttcagcatcttttactttcaccagcgtttctgggtgagcaaaaacaggaaggcaaaatgccgcaaaaaagggaataagggcgacacggaaatgttgaatactcatactcttcctttttcaatattattgaagcatttatcagggttattgtctcatgagcggatacatatttgaatgtatttagaaaaataaacaaataggggttccgcgcacatttccccgaaaagtgccacctgacgtctaagaaaccattattatcatgacattaacctataaaaataggcgtatcacgaggccctttcgtc

SEQ ID NO: 2 - DNA, 19472 bp, Artificial Sequence
  Plasmid 2 - Example 2
tcgcgcgtttcggtgatgacggtgaaaacctctgacacatgcagctcccggagacggtcacagcttgtctgtaagcggatgccgggagcagacaagcccgtcagggcgcgtcagcgggtgttggcgggtgtcggggctggcttaactatgcggcatcagagcagattgtactgagagtgcaccatatgtttgcaaaacgattcaaaacctctttactgccgttattcgctggatttttattgctgtttcatttggttctggcaggaccggcggctgcgagtgctgaaacggcgaacaaatcgaatgagcttacagcaccgtcgatcaaaagcggaaccattcttcatgcatggaattggtcgttcaatacgttaaaacacaatatgaaggatattcatgatgcaggatatacagccattcagacatctccgattaaccaagtaaaggaagggaatcaaggagataaaagcatgtcgaactggtactggctgtatcagccgacatcgtatcaaattggcaaccgttacttaggtactgaacaagaatttaaagaaatgtgtgcagccgctgaagaatatggcataaaggtcattgttgacgcggtcatcaatcataccaccagtgattatgccgcgatttccaatgaggttaagagtattccaaactggacacatggaaacacacaaattaaaaactggtctgatcgatgggatgtcacgcagaattcattgctcgggctgtatgactggaatacacaaaatacacaagtacagtcctatctgaaacggttcttagacagggcattgaatgacggggcagacggttttcgatttgatgccgccaaacatatagagcttccagatgatggcagttacggcagtcaattttggccgaatatcacaaatacatctgcagagttccaatacggagaaatcctgcaggatagtgcctccagagatgctgcatatgcgaattatatggatgtgacagcgtctaactatgggcattccataaggtccgctttaaagaatcgtaatctgggcgtgtcgaatatctcccactatgcatctgatgtgtctgcggacaagctagtgacatgggtagagtcgcatgatacggaattcgagctcggtaccgaactcctttttcatatgagaaggtgccatgtcactattgcttcagaaatactcctagaataaaaaaactcatctttaaagatgagctgtccattccataaaaaattacattgtaatcatgtccagaaaatgatcaatcacaatggaggacattcctaatgccggtgcattctgtcctaaggaagatggcaataattcatagctattgcctaattgggaataaacccttgatgatacttcacttctcattgaatttaaaaccataggatgcgattcaattatgctatttcttaaaattacggcttgtgggttgaaagtatttagaatattggtaaggcctattcctaaatagaatccaaaattttgtaatgcatttaaggttccgatatcattcagatgggcgaggtttatgatatcttgataggacagttttttctctttggtctgaagagattttaataaagccttctctgaagcatacaattcccagcatcctcggtttccgcaactgcatttaggaccattaaagtctattgtcatatgtcccatttctccagagaagccgcttactcctctatataaatgattgttgataataacaccgatccctattcctgtgctgatacttacgtaaataatgttatcgtgattttttgcagctccaaatactttttctccatatgcgccagcatttgcctcattttcaataaaaacaggcacattgtacttctcttgtatcgaagattttaagtcaatatctctccagttggagttcggagtgaaaacaattttttgatctttatcaatgagtccaggcacgcaaatacctataccaataagcccgtacggagattggggcatttgcgtaataaagtgatgaatcatatcaatcaaaatgtctttcgttatttctggagaattggattccaaatggcggtattgatcaagaacgattgttccttcaaggtctgttaaaatgccattaatataatccacaccaacatctattccaacggagtatcctgcctttttattaaaaacaagcatgacaggtcttcttccgccacttgattgtccttgacctatttcaaataccatactttctttcattaacgtgtttacctgtgatgagacagttgatttatttaatccagtcatttcagataattttgctcttgaaataggtgaatttttaaggatttcttttaataataacttttgatttacttttttgacaaaggtttgatcagcgatatccacttcatccactccatttgtttaatctttaaattaagtatcaacatagtacatagcgaatcttccctttattatatctaatgtgttcataaaaaactaaaaaaaatattgaaaatactgacgaggttatataagatgaaaataagttagtttgtttaaacaacaaactaataggtgatgtacttactatatgaaataaaatgcatctgtatttgaatgaatttatttttaagggggaaatcacatggctcaatctcattccagttcaatcaactattttggaagcgcaaacaaagtggtttactaaggtacccgggctagctttaagaaggagatatacatatgagtgaaattaaaaaagcattaaatacgcttgaaattgaagattttgatgcaattgaaatggttgatgttgatgctatgccagaaaacgaagcgcttgaaattatgggagcgtcatgtacgacatgcgtatgtacatgcagttgttgtacaacttaatctagctttaagaaggagatatacatatgagtgaaattaaaaaagcattaaatacgcttgaaattgaagattttgatgcaattgaaatggttgatgttgatgctatgccagaaaacgaagcgcttgaaattatgggagcgtcatgtacgacatgcgtatgtacatgcagttgttgtacaacttaatctagctttaagaaggagatatacatatgagtgaaattaaaaaagcattaaatacgcttgaaattgaagattttgatgcaattgaaatggttgatgttgatgctatgccagaaaacgaagcgcttgaaattatgggagcgtcatgtacgacatgcgtatgtacatgcagttgttgtacaacttaatctagctttaagaaggagatatacatatgagtgaaattaaaaaagcattaaatacgcttgaaattgaagattttgatgcaattgaaatggttgatgttgatgctatgccagaaaacgaagcgcttgaaattatgggagcgtcatgtacgacatgcgtatgtacatgcagttgttgtacaacttaacgaataaaactaaaggagaacaattttatgtatgaaaataatgtaaaagatacaaaggatttttataatgatatagggcatataagttggagtgttgccccctcgcaacactatcatgtgggaatttttgaattagaaaaagattccatggaggatgctcaaaatagaacggtagaatatatggcacgtaaagttgcggcatcagatcttgacgtactattagatattggatgtggctccgggcttactgcagtacaaattagtaaaaaggaaaattgtaaaattgtaggtataaatatttccgaaaagcaacttgcaattgggaaaaagctaatttctaaagagaaaattaatagcagggtaaagctaatgaatatggacgcacatcaattaaactttaagtcaggtatgtttgatggtgcatacgctctagagagtatcatgcatatgaatagggaaaaggttttaagtgaggtacatagagtattaaaaaatggtgctccttttagtttatgtgattggtatgtaaagaaatctttaactccagtagagaagaggtttttagaaaccattacacttggtaagtatattacaaaggaacagtattttagtctttatcaaactcaaaatttcatggatattgaaattgaagaatggagcaataaaatattaccgacttataaatattggacgacgattacggatgaaatgaaagaaaaacttcctgatcatttactatatgtaatagaagaaaattctaaagtactatcagatattgcaattgaaaaattaggatatttacaagtgaatggaataaaacgttagctcgagcaccaccaccaccaccactgacgtacgggcccaagcggtacccggggatccgtttgttccctttatagaaaggaatgatcaaatgttagaaataaaagaaaaacaatttattaaattaaaagaggacacattcttttttccttcagctgaagggatatactttaggaattctataggttattttacaatcaaaggtagaaatatttacccgttttttagtgaaatcagtaaatatttgaatggtaaatatactttgaaagatatagtgagtgagttaagcaaaacccaagaagaaaaatttttaaaattaattgccatattagagaagaatggttttgtaaaatataccgaaagggttattgatgaaaattattataaaaattatgaaaaagaaattgcatttatagattattatactaataatggcatcgaattatttaaaaaactctctaatttcaagatttgtttatatggtagcaataagttatctaatactattcaaaaaagcttagaaaacatagggatacaaaatattaaaagaggctctcgttttgattttgagggagacattgttatttattgcaataatgatgttaatgaaagggaaaatctactggaatgtatggacttttctcagaataaaatatttatttttgtaggtaataaagaatcattaggaattattagtcctattataaaaaatttagatgattggaaggaatttgaaaatatattagagattggtgcagataatattaaagaaaatacaacatttactagcaactctatattaagtagtatgctaagttttgaaattataaagtatgtaacaaattgtttgcaaagtgatttaattaatgcggcatacattttaaatactgatactttaaaagggaattttgttcaggtaaaaaaaaaaatagacttaaaacaagattttattgaaactttcaaacaatcaagcggaggcaacggtttgtatatcaataaaataggtagaggttctaggaaacaaattccgctctcgcaatgggaggttgaattggataaattaggtgacatgaatagtgaaaaaattaaggtcgttagctttggtgatacccaccaggaagcgaggtttaatacttattataaaaccatagaacatctaataatcaatggggaatttaacttagaggaatcatatagctttaagaatcttgatacaatcactttagctattgatgaacaatttaaaagaaaattaacaatttcatgcgacatagataaagaacttgcaatcagaaaagcaatattaaaagcaattttaaagagggaaattaatgtaattgataattatcaagagctttccccattaaaaataagtgattatatagataataaaaatatacaatactattgtaaactgattaacattttaaaagcgaaaatagaattgcgttttaagaaattagtagagggtttgtttttggtagtagttagtgacaatagttataggggagttagtataggatttaatttaaatacagcattagaaaatgctcttaggcaatttattaataatttacaaaatagtatctatacaataaatattgaagatgtaatatttaaaagaattaatgattgggatgatgaatgcattcgagagtttttgacagatgaaaaattagaagtttttatctgtagtatacaaaataatgttatttcagcagaaatttctatagttggagcaatattaatagaaagttaggtgaattgaaaaatgaataaggaagtccttataatcagggatgaaagctttggagaattttttgattctttttttttaaatgaaaataatcgaaaagtttgttttatagatagtaataaaaaagatttgaaatatttattaaaaaactttttagagaataaaaagtttagttatgtactaatctttccaaaggaatggaatcctatgatgtataggtcacttgatgcagtgttagaagactatgatgtaccgtggatctatataacacaattttttaataaaattttaataggtccttttagaaattctaagcaaaaaggttgtttagattgtttatattatagatggtttatgacaaaaaaggatcgtattaatttatttgaattgaagaaatgtttatcagaaggacataatgtaaaaatatctggagatttattgaatgcttcaatggttggattagcaattactttagcatttaaactaataaataatgaggtttcggaattttcgtatattattgacaaaaagacattgagattcaatggtcataattttttacctaatccacattgtcaagtatgtgggcacatggataatgacgagaaaagattaatagaacacaaattttttacagcacttaacgataatactcttaaagaaaagaaaggaaatcgttttttatcaaaagaatatttagaagataccctatctaaaaattttttagatgtagaaactggtatatttaataaacttttggacgattatgaaagtcctttcgcagtttcggtagcaaatcttcctttaaaggttggaaaggatgaggttggtgttggaagaacggataattatgctaatagtcacttaactgcaatattagaaggaatagagagatattgcggaatggaaccaagggggaatagaactaacgtttttggtagttataatgagctaatggaaaatgctctcaatccatctgttttaggattacacgcggaagaacagtatcaattaaaaagatttccttttaataaatataatccagataaaaaaatgaaatgggtctgggggtattcttttaataagaataaggcgatattagtccctgaaacttatgcctattatggtacgaattatagagatggcgttcaaaatagttttgtttatgaaatctcgaatggatgtgctttaggaggacatttattggaagctacattgcaaggaatttatgaagtagtggaaagagatgcttttcttatatcttggtatactaaattaccattaaaacgtataagaaaagaatctattaaggatcagacgattcaattattattaacgagatttgaatatcaaactgattatgatattcatctgtataatatgactttagagaataaaataccaactattttagctattgcaaaaaatagaggtgcttttggcatgaatattttatgtgctgcaggttgtcatttagatataaataaagcaattgaaagttcattacatgagttatgtggaatcttagaggcaatcaaaagtaaatttgaaaataggaaaagtgaattatacgaaatggcaaagaattattcacttgtacggacgatggaagatcattcattattatttggattgaaagaacttgaaaaagagtttgattttctattaaagagcccgattgaaattgatttaagtgaggtagaacctttaaaatatagcaacaatatacatacagatttattgaatgtaattgattattttaaaaaaataaatttagatatcatcgtagtcgatcaaaccgcggaagatataaaatttaacaacttgtattgtgtaaaagttattattccaggaatgttacctatgacatttggacatgatatgagaagaatacataatttaccaaggatattccgtgttccaagggaattaggacataaaattaagaatgaaaatgaaattaagaacaatcaggtaactcctcatcctttcccataacattttttatgaaagatggtgatataacatgaaaccaataaactatgtaccacattttttatgtagaatatctggtgaagaaataaactctatttcagaaattgagtttattaaaaccttggaatgtttagaattatccgaaggaattttaaggaaaataaattctttatcagcagacttaacgaaagatttacatgattgtatttctttatataaagaacaatctatttcacgtgtattaataaatcttaaaagagatatttttaatatgaggtttaatcgagttcaaaagtataaactagaaaatatctcaggttttaaccacgataaattaaatttatggttaaatttagctcaagaatatcaaagcacgctacatctgatgagagaaacttttaaaatggaaatacaggaaaaaagagggaaattaaagcagttatttagtaatagtgaatatataaaagccattcaagtctcaaatactcaactttatgaaaatctcctagaatacttacaagataatcaaagtcatcctccaaaaaagatgaggaatattgaacagtctctaattaattacctaagtcgtatgatatttaagccaactcccttcagttcatttacaggattaaattacggtttttttagtcaggaagattcaagttttgaaataaatactaaggaaagcaaaggtcacactcgaataaacatggtttatttaaaaaaaattgaaagaatgttattaaatcgaatatctataaaaaataaatgttatgtttcgttaaatcaaacgataaacgaagaggaaaattatatgttttttcgaagaggtaaagatgggactagtcaagcttttactggtgaagcttttataaagataaaaaagagcgagctcttaaaggagttaattcaatattttgaaggaatatcttcaatgaatatagttgaggttgtatcatttctttccgaaaaaacaaattatgaaactgaagctttatataattacttatttaagttagagaaaatgggagtgttagattttagcttaggtgtgtccgaacaatcggacaattacacgaaagatttgatagaaaacttattggggattaaagattcattagttgaaaaatcggtctcacaccttgtagaaatagaaaaaattcaggcgattttctctgaatccaattaccaaaaacgttatgtacttttaaaaaatttacaagaacatataaagaagatttatagtttatttgatttaaaattagagtctaatgatttgacctctctattattcgaggatgttagttataaaaatactaagattatattaaatgaaaatcaatggaaaacgcatcttgatgattttaatttaattaagaatttaatgccactttttgatgataatatccttgaaaaattaagtatgaatataatttttaaggatatatatggtaacaagggggcaatagatttattagaattctatagagagtttaataaatatgataaaaatttattatggaagaaaattagaaaaaatgatacatatctttatttaaaaaaattgagaacagagttttatgattatctagaaacacaaattaatatggggttagacactatctttttaaataaaagttggttaaagaaatttattaacaagttccctgatttattgaagagtaaggaaaattattctttctattttcaaatagcctatgataatcaagataatagaattttagttttaaataagatagggccaggattaggtaagcacttttcaagatatggtaatttatttttaaatagcgaatacaaggaaaataatagatttattaattctcttatagaacagtataaaaaatatgatcaaaatgggggggttttaacagatttaaatgcagtgttaggtctaaatcttaatatgcatcctaatcttttaaattatgaaattacttatccaggatgcaatcctagtaaaggaattaatcaagtagcattaaaggatattgaagtattgtatgattctaattctgaccaactaaaattatattctaaacaatatagacagaatgttaaattacttccattgggatttttgtttccagcattgtccccatctttatataagtttttatgtggattttcggaatcaaatgggatagagtattctttttggaacaagttcttaaatgaacacaataataatttttcacttttacctagaattatgttaggatcagtagctttggatagaagaacatggaaaattaatgcgaaggaaatacaaaaggaattttctaaagatacatttgaaacttttattaacttccataagtgggtgaaagaaaatcaactaccggaagatatatttttaagggttgcaaacacaatggacgcttttagtgagaatgaattattaaatcaagatttaggaagttggattgcagaaattaaacaaactaaacatcgtaaacctcaatatgttaattttaataattactttcatatcgatgccttaagaaagattattaaagatgttaataatacagtaacaattcaagaagtttatcctcatccagatgatgtgtattatcaaaaaaatagtaaaaaatgtgtagaatttttagttgaggttttttaataaaggaatgattatatgaacgagaataattttatatggaaggcttatcatattttttatcatcaaaatcaagattttctaattacaaattgtatcaaaccaattttagatgaattgataaaaaagaaattaattagtaaatttttttttataagatattgggaaggcggacctcatattagagtgcgactttattgtacattaaataaatctcaagaagttgattataaatttaatgattttgtttctaaattcttgaaaacatatccttcttcatcaacattagatagaaacatgataaagaatcaattagcaaaattagctagtcttgaagagggtactgagtcaacatgtgttcgagagaataatcatattattcatctagaatataatccagagtataaacgatatggaggagaaaatggaatagagattgcggaagaacatttttaccattcaagtataatgtgtttgaagttaatacaagaaattaataaaaagacaaatcgtttgcgcatatctattgaaattatactatcttatttaaaagctatgaatatgaacttacaagagagtattaagtttttagaaggctattatctaatatggaaaagatatgtatacagcaataccaataacgttgaagaattcttcgctaacaaatatattaagcaaaaaaaagtaatagacaaaattgtagtaaactatttcaattctaataataataaaggtatgttaggagaaaaatggagtaatcatttgaatttaactgtacagaatttagaaaatgattgggatcggggagaattaataatagataaagatgttttagcatatataaatatccctcaaaagattgcttttatagttacaagttatgttcatatgacaaacaataggcttggtatcatgccgcaagaagaagcctatttaagctatatgcttttatgtagtttgaaatcattgtataagagtagaaagggatgacttaaatggagcagtatcataaaattgtattaactggaagtaatgctgagactatgttaataaaaaatatagagcctgtagcagttaagtttataaataactataagggttttttctatgtttttaaatatagtaaagattttccaattatcgatgtttatatcaacaacaaaattgttacagaaaatcaattaaataaaattttacagaattctggggctaaatataaaatttataaaaattcaatatttaatgagacacaagggaattttgggatgttaggtgataaatatctggcagaattttttaaaaagacaaatgaaattagccttaatatactaaatcaaaattttgagagttacaataaaaaaatagaatttgcgctagagataatgttaatttcagcgcactataattatgattcaataaaaaaaggctacttatcctatgcatctcatgtaaatggattttttactagatggaaagatccaaataaaattagagatatatttcataagaactacttaaataacaaagagtacctagaatcgaaagtttcagaaataatagataataacaacagaagtagcttgagcgaattatcggatattattacagaaatgaagaaagagatgactactgatattgagaaggggaacctgcatgtatttaatattgaattactacaaaaaccaggagaaagagattttctagaaaaaagtcagtttcataagacgatattaaataatccagatttctctaattttatgaataaagatataaactttttaggttcacgcctaataactgtatttacgtacttattaatacgaaatttagggattcaaaataaagatagatatctactttgctactatatctataaaattattgaagaaaaatataatatagatactttggaattaataagggattttggtaaagggagggataataatgttgaagacttacaaagatattgaagattttttatataatttgcaatattcgcctgctaaagcttcagatttcaatttagatttaagtaattatgatagacccttgccttttaaaatttataggaatagagaatcgatagatttagacgataactttccgatttgtattaatgatttagatggtattgattattcaaatttcgaaattattagttatttattgtggtatacctatggttttaccagctacaattggttaacaaaaccaacattaaatggtcagaatacatccttaagtttttttagaagaagtgtagcctcaggtggcggcttatatcctggggaaatttacttatatgtggagagtattaaaggtatcaagtcaggattatattattttgatgttaggggaccgagattaattttactaagggaaggaaattttcaagaatttatcaaaaaatctttgcaatataatcaagatagaaatgtttatatttttataacatcattttattggaaaaacttctttaaatatttaaatttctcgtatcgtttacaaggcttagatatcggtgctattgtaagccaagctcacctaatttcaaagaaattaggtcttaattcggagattaggtatcactttgatgataaaaaaattaatgattttttaggaatcaacgctgaggaagaaagcagctacgtagttttgcctatagatatggataataattcatataaaagtgaaaataaggttcccgcttttgagtactttaaaaacgatacaacattcaattatattgaacatttaaatgttggccccaaaaatgtatgtcaggatatttataaaatcaatagtaatattatcaatagtggcttaattaaagttaaaaaaaatgaaatagcatcttttaaagaggaggcaaatgttgttcataaagaaaaatatgattatgacattttgaaggcttctgtaagtcgtatatcaccaggagagaactttttgtctgattttttgaatattcagcatgttcacaaagttctagatgttggaatgcaggaacaatttaaaaatgatatttttagcgataattatagtgttctaaaggatgttgaaatttacttttatgccaataagattgaaggtttaccaaaaggctactattactataatccaagtaataaaagtttcgttttgaaacataaaggtgatttttctagtgtttttcaggagaatcttacacgaaaaaattttaatttagtagaaatgcctttaattgtgcacttagtattaaacatgaaaaaatttatagaaaatatgaaatttagaggctatagagtcatgcaaatggaggcagggagaattatgcatcaaatacaattgaatgctgcaggtttgaacctagggagccatccaatgttaggttatagggctgataatttggaggagttttttggtattcaaaataatataactgtccagatgtctattggtaaatatagacctttattgaggctaaccaataatttattgaataaaactaaaggagaacaattttatgtatgacggaaaacgggtgaatccatatgaactctatcaaacaatttaattttaaaaataaaaatatttttattactggagctaccagtgatatagctatctgtatagcagaatccttctctggatttggcgggaatttaattttatctgatactgataaacaattaccaaaattagaacatgttaaacaaaaaatgattgaaaaatttaggaataatgttcaaattgtaactattgatttatataaggttaatgatatacaaaatgcaattgaaaaattagataaaccaattgatatattgatcaattgtgctggaaataattactttgttccagctctggaggttagtgaagagaattggcaaaaaattatagatgtaaatttgaaaggaactttttttcttagtcagtcaatagcaaaaaaaatgattagtgacggcataaaggggaaaattgtaaatattggatcgcaacatggggtagttgccaatggtctaagagccccctattgtattagtaagtttggattaataggtttgacaaaagttttagcgctagagtggtctacttttaatatattggttaattgtgtttcaccaacgtatgtaaaaacttctaaaagtaaggatttcttggagcatgaagatgttaaaaaagcatatttatataaaatccctttgaaaaaatatgctttaccccacgatatatcatatgcagtattgtttttaagtagcgatcaaaatcagataattacaggggaaaatattttagttaatggtggttatacattacactagatctcaccaccaccaccaccactgacgtacgggcccaagcttgcacccattagttcaacaaacgaaaattggataaagtgggatatttttaaaatatatatttatgttacagtaatattgacttttaaaaaaggattgattctaatgaagaaagcagacaagtaagcctcctaaattcactttagataaaaatttaggaggcatatcaaatgaactttaataaaattgatttagacaattggaagagaaaagagatatttaatcattatttgaaccaacaaacgacttttagtataaccacagaaattgatattagtgttttataccgaaacataaaacaagaaggatataaattttaccctgcatttattttcttagtgacaagggtgataaactcaaatacagcttttagaactggttacaatagcgacggagagttaggttattgggataagttagagccactttatacaatttttgatggtgtatctaaaacattctctggtatttggactcctgtaaagaatgacttcaaagagttttatgatttatacctttctgatgtagagaaatataatggttcggggaaattgtttcccaaaacacctatacctgaaaatgctttttctctttctattattccatggacttcatttactgggtttaacttaaatatcaataataatagtaattaccttctacccattattacagcaggaaaattcattaataaaggtaattcaatatatttaccgctatctttacaggtacatcattctgtttgtgatggttatcatgcaggattgtttatgaactctattcaggaattgtcagataggcctaatgactggcttttataatatgagataatgccgactgtactttttacagtcggttttctaatgtcactaacctgccccgttagttgaagaaggtttttatattacagctccagatcctctacgccggacgcatcgtggccggcatcaccggcgccacaggtgcggttgctggcgcctatatcgccgacatcaccgatggggaagatcgggctcgccacttcgggctcatgagcgcttgtttcggcgtgggtatggtggcaggccccgtggccgggggactgttgggcgccatctccttgcatgcaccattccttgcggcggcggtgctcaacggcctcaacctactactgggctgcttcctaatgcaggagtcgcataagggagagcgtcgacatggatgagcgatgatgatatccgtttaggctgggcggtgatagcttctcgttcaggcagtacgcctcttttcttttccagacctgagggaggcggaaatggtgtgaggttcccggggaaaagccaaataggcgatcgcgggagtgctttatttgaagatcaggctatcactgcggtcaatagatttcacaatgtgatggctggacagcctgaggaactctcgaacccgaatggaaacaaccagatatttatgaatcagcgcggctcacatggcgttgtgctggcaaatgcaggttcatcctctgtctctatcaatacggcaacaaaattgcctgatggcaggtatgacaataaagctggagcgggttcatttcaagtgaacgatggtaaactgacaggcacgatcaatgccaggtctgtagctgtgctttatcctgatgatattgcaaaagcgcctcatgttttccttgagaattacaaaacaggtgtaacacattctttcaatgatcaactgacgattaccttgcgtgcagatgcgaatacaacaaaagccgtttatcaaatcaataatggaccagacgacaggcgtttaaggatggagatcaattcacaatcggaaaaggagatccaatttggcaaaacatacaccatcatgttaaaaggaacgaacagtgatggtgtaacgaggaccgagaaatacagttttgttaaaagagatccagcgtcggccaaaaccatcggctatcaaaatccgaatcattggagccaggtaaatgcttatatctataaacatgatgggagccgagtaattgaattgaccggatcttggcctggaaaaccaatgactaaaaatgcagacggaatttacacgctgacgctgcctgcggacacggatacaaccaacgcaaaagtgatttttaataatggcagcgcccaagtgcccggtcagaatcagcctggctttgattacgtgctaaatggtttatataatgactcgggcttaagcggttctcttccccattgatagcttggcgtaatcatggtcatagctgtttcctgtgtgaaattgttatccgctcacaattccacacaacatacgagccggaagcataaagtgtaaagcctggggtgcctaatgagtgagctaactcacattaattgcgttgcgctcactgcccgctttccagtcgggaaacctgtcgtgccagctgcattaatgaatcggccaacgcgcggggagaggcggtttgcgtattgggcgctcttccgcttcctcgctcactgactcgctgcgctcggtcgttcggctgcggcgagcggtatcagctcactcaaaggcggtaatacggttatccacagaatcaggggataacgcaggaaagaacatgtgagcaaaaggccagcaaaaggccaggaaccgtaaaaaggccgcgttgctggcgtttttccataggctccgcccccctgacgagcatcacaaaaatcgacgctcaagtcagaggtggcgaaacccgacaggactataaagataccaggcgtttccccctggaagctccctcgtgcgctctcctgttccgaccctgccgcttaccggatacctgtccgcctttctcccttcgggaagcgtggcgctttctcatagctcacgctgtaggtatctcagttcggtgtaggtcgttcgctccaagctgggctgtgtgcacgaaccccccgttcagcccgaccgctgcgccttatccggtaactatcgtcttgagtccaacccggtaagacacgacttatcgccactggcagcagccactggtaacaggattagcagagcgaggtatgtaggcggtgctacagagttcttgaagtggtggcctaactacggctacactagaagaacagtatttggtatctgcgctctgctgaagccagttaccttcggaaaaagagttggtagctcttgatccggcaaacaaaccaccgctggtagcggtggtttttttgtttgcaagcagcagattacgcgcagaaaaaaaggatctcaagaagatcctttgatcttttctacggggtctgacgctcagtggaacgaaaactcacgttaagggattttggtcatgagattatcaaaaaggatcttcacctagatccttttaaattaaaaatgaagttttaaatcaatctaaagtatatatgagtaaacttggtctgacagttaccaatgcttaatcagtgaggcacctatctcagcgatctgtctatttcgttcatccatagttgcctgactccccgtcgtgtagataactacgatacgggagggcttaccatctggccccagtgctgcaatgataccgcgagacccacgctcaccggctccagatttatcagcaataaaccagccagccggaagggccgagcgcagaagtggtcctgcaactttatccgcctccatccagtctattaattgttgccgggaagctagagtaagtagttcgccagttaatagtttgcgcaacgttgttgccattgctacaggcatcgtggtgtcacgctcgtcgtttggtatggcttcattcagctccggttcccaacgatcaaggcgagttacatgatcccccatgttgtgcaaaaaagcggttagctccttcggtcctccgatcgttgtcagaagtaagttggccgcagtgttatcactcatggttatggcagcactgcataattctcttactgtcatgccatccgtaagatgcttttctgtgactggtgagtactcaaccaagtcattctgagaatagtgtatgcggcgaccgagttgctcttgcccggcgtcaatacgggataataccgcgccacatagcagaactttaaaagtgctcatcattggaaaacgttcttcggggcgaaaactctcaaggatcttaccgctgttgagatccagttcgatgtaacccactcgtgcacccaactgatcttcagcatcttttactttcaccagcgtttctgggtgagcaaaaacaggaaggcaaaatgccgcaaaaaagggaataagggcgacacggaaatgttgaatactcatactcttcctttttcaatattattgaagcatttatcagggttattgtctcatgagcggatacatatttgaatgtatttagaaaaataaacaaataggggttccgcgcacatttccccgaaaagtgccacctgacgtctaagaaaccattattatcatgacattaacctataaaaataggcgtatcacgaggccctttcgtc

SEQ ID NO: 3 - DNA, 19738 bp, Artificial Sequence
  Plasmid 3 - Example 2
tcgcgcgtttcggtgatgacggtgaaaacctctgacacatgcagctcccggagacggtcacagcttgtctgtaagcggatgccgggagcagacaagcccgtcagggcgcgtcagcgggtgttggcgggtgtcggggctggcttaactatgcggcatcagagcagattgtactgagagtgcaccatatgtttgcaaaacgattcaaaacctctttactgccgttattcgctggatttttattgctgtttcatttggttctggcaggaccggcggctgcgagtgctgaaacggcgaacaaatcgaatgagcttacagcaccgtcgatcaaaagcggaaccattcttcatgcatggaattggtcgttcaatacgttaaaacacaatatgaaggatattcatgatgcaggatatacagccattcagacatctccgattaaccaagtaaaggaagggaatcaaggagataaaagcatgtcgaactggtactggctgtatcagccgacatcgtatcaaattggcaaccgttacttaggtactgaacaagaatttaaagaaatgtgtgcagccgctgaagaatatggcataaaggtcattgttgacgcggtcatcaatcataccaccagtgattatgccgcgatttccaatgaggttaagagtattccaaactggacacatggaaacacacaaattaaaaactggtctgatcgatgggatgtcacgcagaattcattgctcgggctgtatgactggaatacacaaaatacacaagtacagtcctatctgaaacggttcttagacagggcattgaatgacggggcagacggttttcgatttgatgccgccaaacatatagagcttccagatgatggcagttacggcagtcaattttggccgaatatcacaaatacatctgcagagttccaatacggagaaatcctgcaggatagtgcctccagagatgctgcatatgcgaattatatggatgtgacagcgtctaactatgggcattccataaggtccgctttaaagaatcgtaatctgggcgtgtcgaatatctcccactatgcatctgatgtgtctgcggacaagctagtgacatgggtagagtcgcatgatacggaattcgagctcggtaccgaactcctttttcatatgagaaggtgccatgtcactattgcttcagaaatactcctagaataaaaaaactcatctttaaagatgagctgtccattccataaaaaattacattgtaatcatgtccagaaaatgatcaatcacaatggaggacattcctaatgccggtgcattctgtcctaaggaagatggcaataattcatagctattgcctaattgggaataaacccttgatgatacttcacttctcattgaatttaaaaccataggatgcgattcaattatgctatttcttaaaattacggcttgtgggttgaaagtatttagaatattggtaaggcctattcctaaatagaatccaaaattttgtaatgcatttaaggttccgatatcattcagatgggcgaggtttatgatatcttgataggacagttttttctctttggtctgaagagattttaataaagccttctctgaagcatacaattcccagcatcctcggtttccgcaactgcatttaggaccattaaagtctattgtcatatgtcccatttctccagagaagccgcttactcctctatataaatgattgttgataataacaccgatccctattcctgtgctgatacttacgtaaataatgttatcgtgattttttgcagctccaaatactttttctccatatgcgccagcatttgcctcattttcaataaaaacaggcacattgtacttctcttgtatcgaagattttaagtcaatatctctccagttggagttcggagtgaaaacaattttttgatctttatcaatgagtccaggcacgcaaatacctataccaataagcccgtacggagattggggcatttgcgtaataaagtgatgaatcatatcaatcaaaatgtctttcgttatttctggagaattggattccaaatggcggtattgatcaagaacgattgttccttcaaggtctgttaaaatgccattaatataatccacaccaacatctattccaacggagtatcctgcctttttattaaaaacaagcatgacaggtcttcttccgccacttgattgtccttgacctatttcaaataccatactttctttcattaacgtgtttacctgtgatgagacagttgatttatttaatccagtcatttcagataattttgctcttgaaataggtgaatttttaaggatttcttttaataataacttttgatttacttttttgacaaaggtttgatcagcgatatccacttcatccactccatttgtttaatctttaaattaagtatcaacatagtacatagcgaatcttccctttattatatctaatgtgttcataaaaaactaaaaaaaatattgaaaatactgacgaggttatataagatgaaaataagttagtttgtttaaacaacaaactaataggtgatgtacttactatatgaaataaaatgcatctgtatttgaatgaatttatttttaagggggaaatcacatggctcaatctcattccagttcaatcaactattttggaagcgcaaacaaagtggtttactaaggtacccgggctagctttaagaaggagatatacatatgagtgaaattaaaaaagcattaaatacgcttgaaattgaagattttgatgcaattgaaatggttgatgttgatgctatgccagaaaacgaagcgcttgaaattatgggagcgtcatgtacgacatgcgtatgtacatgcagttgttgtacaacttaatctagctttaagaaggagatatacatatgagtgaaattaaaaaagcattaaatacgcttgaaattgaagattttgatgcaattgaaatggttgatgttgatgctatgccagaaaacgaagcgcttgaaattatgggagcgtcatgtacgacatgcgtatgtacatgcagttgttgtacaacttaatctagctttaagaaggagatatacatatgagtgaaattaaaaaagcattaaatacgcttgaaattgaagattttgatgcaattgaaatggttgatgttgatgctatgccagaaaacgaagcgcttgaaattatgggagcgtcatgtacgacatgcgtatgtacatgcagttgttgtacaacttaatctagctttaagaaggagatatacatatgagtgaaattaaaaaagcattaaatacgcttgaaattgaagattttgatgcaattgaaatggttgatgttgatgctatgccagaaaacgaagcgcttgaaattatgggagcgtcatgtacgacatgcgtatgtacatgcagttgttgtacaacttaacaattagagaggagtatacatatgcttactgaaaaacaagtaaacttttttaaaaaaaatggttatctaattttagaagattttttttctttacatgaactaaaacaaatgaaattaacatttcaacataagataaaaaatcaaaagaactcaaaaggattctattcaggcatcttaactcaacaccttaatctttggaataaggattctttttttaagaaccttgtatttaacaaaagaatttcgagaattgcaaaagaactgttggagactaagaatatacggattttacaagatcatgccttaattaaaaaaagcatagtaggtaaagctactccttggcatcaggatttctcttattttccaattaatgaacctgaagcattaactgtttggattccgtttcaagatgtctatgaaaaaaatggatgtatgagctatcttcctacttcaaatacattaggaagattaactaaagttcatatgtataatatcgataaacctttagaagatataaacatttctcctgcgatagctaaactaaaagctgggagtatagttattcatcattctttaactttgcattatgcatactctaacataagtgataatgatcggttggcctatgcaattgtctatatgaaagatgaagtaacttataatggaaacagacatccactgatagataaaaatttatttgccaaaaatcaaaaattagaagggaccaacttccctattatcgaggagagtgtaacgttaacatgataaaagaacttgatcacgtaatgataaaagtccaaaatctagaagaaagtattactttttattcagagcagttacgactgcaaataatctgggagtatgataattatgtaggatttcataacggtatagttattcatgattcgaaaaacagtgaaaatttaactagctttttcaaagtagattctgtagaagaaacagtcaaaatattaaaagagagcaatgttaaaattattttagagcccactcctattccgactggatatacagcagcctttcaagacatcagtaataacattattcatattgtagataatattaatctttcttgactcgagcaccaccaccaccaccactgacgtacgggcccaagcggtacccggggatccgtttgttccctttatagaaaggaatgatcaaatgttagaaataaaagaaaaacaatttattaaattaaaagaggacacattcttttttccttcagctgaagggatatactttaggaattctataggttattttacaatcaaaggtagaaatatttacccgttttttagtgaaatcagtaaatatttgaatggtaaatatactttgaaagatatagtgagtgagttaagcaaaacccaagaagaaaaatttttaaaattaattgccatattagagaagaatggttttgtaaaatataccgaaagggttattgatgaaaattattataaaaattatgaaaaagaaattgcatttatagattattatactaataatggcatcgaattatttaaaaaactctctaatttcaagatttgtttatatggtagcaataagttatctaatactattcaaaaaagcttagaaaacatagggatacaaaatattaaaagaggctctcgttttgattttgagggagacattgttatttattgcaataatgatgttaatgaaagggaaaatctactggaatgtatggacttttctcagaataaaatatttatttttgtaggtaataaagaatcattaggaattattagtcctattataaaaaatttagatgattggaaggaatttgaaaatatattagagattggtgcagataatattaaagaaaatacaacatttactagcaactctatattaagtagtatgctaagttttgaaattataaagtatgtaacaaattgtttgcaaagtgatttaattaatgcggcatacattttaaatactgatactttaaaagggaattttgttcaggtaaaaaaaaaaatagacttaaaacaagattttattgaaactttcaaacaatcaagcggaggcaacggtttgtatatcaataaaataggtagaggttctaggaaacaaattccgctctcgcaatgggaggttgaattggataaattaggtgacatgaatagtgaaaaaattaaggtcgttagctttggtgatacccaccaggaagcgaggtttaatacttattataaaaccatagaacatctaataatcaatggggaatttaacttagaggaatcatatagctttaagaatcttgatacaatcactttagctattgatgaacaatttaaaagaaaattaacaatttcatgcgacatagataaagaacttgcaatcagaaaagcaatattaaaagcaattttaaagagggaaattaatgtaattgataattatcaagagctttccccattaaaaataagtgattatatagataataaaaatatacaatactattgtaaactgattaacattttaaaagcgaaaatagaattgcgttttaagaaattagtagagggtttgtttttggtagtagttagtgacaatagttataggggagttagtataggatttaatttaaatacagcattagaaaatgctcttaggcaatttattaataatttacaaaatagtatctatacaataaatattgaagatgtaatatttaaaagaattaatgattgggatgatgaatgcattcgagagtttttgacagatgaaaaattagaagtttttatctgtagtatacaaaataatgttatttcagcagaaatttctatagttggagcaatattaatagaaagttaggtgaattgaaaaatgaataaggaagtccttataatcagggatgaaagctttggagaattttttgattctttttttttaaatgaaaataatcgaaaagtttgttttatagatagtaataaaaaagatttgaaatatttattaaaaaactttttagagaataaaaagtttagttatgtactaatctttccaaaggaatggaatcctatgatgtataggtcacttgatgcagtgttagaagactatgatgtaccgtggatctatataacacaattttttaataaaattttaataggtccttttagaaattctaagcaaaaaggttgtttagattgtttatattatagatggtttatgacaaaaaaggatcgtattaatttatttgaattgaagaaatgtttatcagaaggacataatgtaaaaatatctggagatttattgaatgcttcaatggttggattagcaattactttagcatttaaactaataaataatgaggtttcggaattttcgtatattattgacaaaaagacattgagattcaatggtcataattttttacctaatccacattgtcaagtatgtgggcacatggataatgacgagaaaagattaatagaacacaaattttttacagcacttaacgataatactcttaaagaaaagaaaggaaatcgttttttatcaaaagaatatttagaagataccctatctaaaaattttttagatgtagaaactggtatatttaataaacttttggacgattatgaaagtcctttcgcagtttcggtagcaaatcttcctttaaaggttggaaaggatgaggttggtgttggaagaacggataattatgctaatagtcacttaactgcaatattagaaggaatagagagatattgcggaatggaaccaagggggaatagaactaacgtttttggtagttataatgagctaatggaaaatgctctcaatccatctgttttaggattacacgcggaagaacagtatcaattaaaaagatttccttttaataaatataatccagataaaaaaatgaaatgggtctgggggtattcttttaataagaataaggcgatattagtccctgaaacttatgcctattatggtacgaattatagagatggcgttcaaaatagttttgtttatgaaatctcgaatggatgtgctttaggaggacatttattggaagctacattgcaaggaatttatgaagtagtggaaagagatgcttttcttatatcttggtatactaaattaccattaaaacgtataagaaaagaatctattaaggatcagacgattcaattattattaacgagatttgaatatcaaactgattatgatattcatctgtataatatgactttagagaataaaataccaactattttagctattgcaaaaaatagaggtgcttttggcatgaatattttatgtgctgcaggttgtcatttagatataaataaagcaattgaaagttcattacatgagttatgtggaatcttagaggcaatcaaaagtaaatttgaaaataggaaaagtgaattatacgaaatggcaaagaattattcacttgtacggacgatggaagatcattcattattatttggattgaaagaacttgaaaaagagtttgattttctattaaagagcccgattgaaattgatttaagtgaggtagaacctttaaaatatagcaacaatatacatacagatttattgaatgtaattgattattttaaaaaaataaatttagatatcatcgtagtcgatcaaaccgcggaagatataaaatttaacaacttgtattgtgtaaaagttattattccaggaatgttacctatgacatttggacatgatatgagaagaatacataatttaccaaggatattccgtgttccaagggaattaggacataaaattaagaatgaaaatgaaattaagaacaatcaggtaactcctcatcctttcccataacattttttatgaaagatggtgatataacatgaaaccaataaactatgtaccacattttttatgtagaatatctggtgaagaaataaactctatttcagaaattgagtttattaaaaccttggaatgtttagaattatccgaaggaattttaaggaaaataaattctttatcagcagacttaacgaaagatttacatgattgtatttctttatataaagaacaatctatttcacgtgtattaataaatcttaaaagagatatttttaatatgaggtttaatcgagttcaaaagtataaactagaaaatatctcaggttttaaccacgataaattaaatttatggttaaatttagctcaagaatatcaaagcacgctacatctgatgagagaaacttttaaaatggaaatacaggaaaaaagagggaaattaaagcagttatttagtaatagtgaatatataaaagccattcaagtctcaaatactcaactttatgaaaatctcctagaatacttacaagataatcaaagtcatcctccaaaaaagatgaggaatattgaacagtctctaattaattacctaagtcgtatgatatttaagccaactcccttcagttcatttacaggattaaattacggtttttttagtcaggaagattcaagttttgaaataaatactaaggaaagcaaaggtcacactcgaataaacatggtttatttaaaaaaaattgaaagaatgttattaaatcgaatatctataaaaaataaatgttatgtttcgttaaatcaaacgataaacgaagaggaaaattatatgttttttcgaagaggtaaagatgggactagtcaagcttttactggtgaagcttttataaagataaaaaagagcgagctcttaaaggagttaattcaatattttgaaggaatatcttcaatgaatatagttgaggttgtatcatttctttccgaaaaaacaaattatgaaactgaagctttatataattacttatttaagttagagaaaatgggagtgttagattttagcttaggtgtgtccgaacaatcggacaattacacgaaagatttgatagaaaacttattggggattaaagattcattagttgaaaaatcggtctcacaccttgtagaaatagaaaaaattcaggcgattttctctgaatccaattaccaaaaacgttatgtacttttaaaaaatttacaagaacatataaagaagatttatagtttatttgatttaaaattagagtctaatgatttgacctctctattattcgaggatgttagttataaaaatactaagattatattaaatgaaaatcaatggaaaacgcatcttgatgattttaatttaattaagaatttaatgccactttttgatgataatatccttgaaaaattaagtatgaatataatttttaaggatatatatggtaacaagggggcaatagatttattagaattctatagagagtttaataaatatgataaaaatttattatggaagaaaattagaaaaaatgatacatatctttatttaaaaaaattgagaacagagttttatgattatctagaaacacaaattaatatggggttagacactatctttttaaataaaagttggttaaagaaatttattaacaagttccctgatttattgaagagtaaggaaaattattctttctattttcaaatagcctatgataatcaagataatagaattttagttttaaataagatagggccaggattaggtaagcacttttcaagatatggtaatttatttttaaatagcgaatacaaggaaaataatagatttattaattctcttatagaacagtataaaaaatatgatcaaaatgggggggttttaacagatttaaatgcagtgttaggtctaaatcttaatatgcatcctaatcttttaaattatgaaattacttatccaggatgcaatcctagtaaaggaattaatcaagtagcattaaaggatattgaagtattgtatgattctaattctgaccaactaaaattatattctaaacaatatagacagaatgttaaattacttccattgggatttttgtttccagcattgtccccatctttatataagtttttatgtggattttcggaatcaaatgggatagagtattctttttggaacaagttcttaaatgaacacaataataatttttcacttttacctagaattatgttaggatcagtagctttggatagaagaacatggaaaattaatgcgaaggaaatacaaaaggaattttctaaagatacatttgaaacttttattaacttccataagtgggtgaaagaaaatcaactaccggaagatatatttttaagggttgcaaacacaatggacgcttttagtgagaatgaattattaaatcaagatttaggaagttggattgcagaaattaaacaaactaaacatcgtaaacctcaatatgttaattttaataattactttcatatcgatgccttaagaaagattattaaagatgttaataatacagtaacaattcaagaagtttatcctcatccagatgatgtgtattatcaaaaaaatagtaaaaaatgtgtagaatttttagttgaggttttttaataaaggaatgattatatgaacgagaataattttatatggaaggcttatcatattttttatcatcaaaatcaagattttctaattacaaattgtatcaaaccaattttagatgaattgataaaaaagaaattaattagtaaatttttttttataagatattgggaaggcggacctcatattagagtgcgactttattgtacattaaataaatctcaagaagttgattataaatttaatgattttgtttctaaattcttgaaaacatatccttcttcatcaacattagatagaaacatgataaagaatcaattagcaaaattagctagtcttgaagagggtactgagtcaacatgtgttcgagagaataatcatattattcatctagaatataatccagagtataaacgatatggaggagaaaatggaatagagattgcggaagaacatttttaccattcaagtataatgtgtttgaagttaatacaagaaattaataaaaagacaaatcgtttgcgcatatctattgaaattatactatcttatttaaaagctatgaatatgaacttacaagagagtattaagtttttagaaggctattatctaatatggaaaagatatgtatacagcaataccaataacgttgaagaattcttcgctaacaaatatattaagcaaaaaaaagtaatagacaaaattgtagtaaactatttcaattctaataataataaaggtatgttaggagaaaaatggagtaatcatttgaatttaactgtacagaatttagaaaatgattgggatcggggagaattaataatagataaagatgttttagcatatataaatatccctcaaaagattgcttttatagttacaagttatgttcatatgacaaacaataggcttggtatcatgccgcaagaagaagcctatttaagctatatgcttttatgtagtttgaaatcattgtataagagtagaaagggatgacttaaatggagcagtatcataaaattgtattaactggaagtaatgctgagactatgttaataaaaaatatagagcctgtagcagttaagtttataaataactataagggttttttctatgtttttaaatatagtaaagattttccaattatcgatgtttatatcaacaacaaaattgttacagaaaatcaattaaataaaattttacagaattctggggctaaatataaaatttataaaaattcaatatttaatgagacacaagggaattttgggatgttaggtgataaatatctggcagaattttttaaaaagacaaatgaaattagccttaatatactaaatcaaaattttgagagttacaataaaaaaatagaatttgcgctagagataatgttaatttcagcgcactataattatgattcaataaaaaaaggctacttatcctatgcatctcatgtaaatggattttttactagatggaaagatccaaataaaattagagatatatttcataagaactacttaaataacaaagagtacctagaatcgaaagtttcagaaataatagataataacaacagaagtagcttgagcgaattatcggatattattacagaaatgaagaaagagatgactactgatattgagaaggggaacctgcatgtatttaatattgaattactacaaaaaccaggagaaagagattttctagaaaaaagtcagtttcataagacgatattaaataatccagatttctctaattttatgaataaagatataaactttttaggttcacgcctaataactgtatttacgtacttattaatacgaaatttagggattcaaaataaagatagatatctactttgctactatatctataaaattattgaagaaaaatataatatagatactttggaattaataagggattttggtaaagggagggataataatgttgaagacttacaaagatattgaagattttttatataatttgcaatattcgcctgctaaagcttcagatttcaatttagatttaagtaattatgatagacccttgccttttaaaatttataggaatagagaatcgatagatttagacgataactttccgatttgtattaatgatttagatggtattgattattcaaatttcgaaattattagttatttattgtggtatacctatggttttaccagctacaattggttaacaaaaccaacattaaatggtcagaatacatccttaagtttttttagaagaagtgtagcctcaggtggcggcttatatcctggggaaatttacttatatgtggagagtattaaaggtatcaagtcaggattatattattttgatgttaggggaccgagattaattttactaagggaaggaaattttcaagaatttatcaaaaaatctttgcaatataatcaagatagaaatgtttatatttttataacatcattttattggaaaaacttctttaaatatttaaatttctcgtatcgtttacaaggcttagatatcggtgctattgtaagccaagctcacctaatttcaaagaaattaggtcttaattcggagattaggtatcactttgatgataaaaaaattaatgattttttaggaatcaacgctgaggaagaaagcagctacgtagttttgcctatagatatggataataattcatataaaagtgaaaataaggttcccgcttttgagtactttaaaaacgatacaacattcaattatattgaacatttaaatgttggccccaaaaatgtatgtcaggatatttataaaatcaatagtaatattatcaatagtggcttaattaaagttaaaaaaaatgaaatagcatcttttaaagaggaggcaaatgttgttcataaagaaaaatatgattatgacattttgaaggcttctgtaagtcgtatatcaccaggagagaactttttgtctgattttttgaatattcagcatgttcacaaagttctagatgttggaatgcaggaacaatttaaaaatgatatttttagcgataattatagtgttctaaaggatgttgaaatttacttttatgccaataagattgaaggtttaccaaaaggctactattactataatccaagtaataaaagtttcgttttgaaacataaaggtgatttttctagtgtttttcaggagaatcttacacgaaaaaattttaatttagtagaaatgcctttaattgtgcacttagtattaaacatgaaaaaatttatagaaaatatgaaatttagaggctatagagtcatgcaaatggaggcagggagaattatgcatcaaatacaattgaatgctgcaggtttgaacctagggagccatccaatgttaggttatagggctgataatttggaggagttttttggtattcaaaataatataactgtccagatgtctattggtaaatatagacctttattgaggctaaccaataatttattgaataaaactaaaggagaacaattttatgtatgacggaaaacgggtgaatccatatgaactctatcaaacaatttaattttaaaaataaaaatatttttattactggagctaccagtgatatagctatctgtatagcagaatccttctctggatttggcgggaatttaattttatctgatactgataaacaattaccaaaattagaacatgttaaacaaaaaatgattgaaaaatttaggaataatgttcaaattgtaactattgatttatataaggttaatgatatacaaaatgcaattgaaaaattagataaaccaattgatatattgatcaattgtgctggaaataattactttgttccagctctggaggttagtgaagagaattggcaaaaaattatagatgtaaatttgaaaggaactttttttcttagtcagtcaatagcaaaaaaaatgattagtgacggcataaaggggaaaattgtaaatattggatcgcaacatggggtagttgccaatggtctaagagccccctattgtattagtaagtttggattaataggtttgacaaaagttttagcgctagagtggtctacttttaatatattggttaattgtgtttcaccaacgtatgtaaaaacttctaaaagtaaggatttcttggagcatgaagatgttaaaaaagcatatttatataaaatccctttgaaaaaatatgctttaccccacgatatatcatatgcagtattgtttttaagtagcgatcaaaatcagataattacaggggaaaatattttagttaatggtggttatacattacactagtcaccaccaccaccaccactgacgtacgggcccaagcttgcacccattagttcaacaaacgaaaattggataaagtgggatatttttaaaatatatatttatgttacagtaatattgacttttaaaaaaggattgattctaatgaagaaagcagacaagtaagcctcctaaattcactttagataaaaatttaggaggcatatcaaatgaactttaataaaattgatttagacaattggaagagaaaagagatatttaatcattatttgaaccaacaaacgacttttagtataaccacagaaattgatattagtgttttataccgaaacataaaacaagaaggatataaattttaccctgcatttattttcttagtgacaagggtgataaactcaaatacagcttttagaactggttacaatagcgacggagagttaggttattgggataagttagagccactttatacaatttttgatggtgtatctaaaacattctctggtatttggactcctgtaaagaatgacttcaaagagttttatgatttatacctttctgatgtagagaaatataatggttcggggaaattgtttcccaaaacacctatacctgaaaatgctttttctctttctattattccatggacttcatttactgggtttaacttaaatatcaataataatagtaattaccttctacccattattacagcaggaaaattcattaataaaggtaattcaatatatttaccgctatctttacaggtacatcattctgtttgtgatggttatcatgcaggattgtttatgaactctattcaggaattgtcagataggcctaatgactggcttttataatatgagataatgccgactgtactttttacagtcggttttctaatgtcactaacctgccccgttagttgaagaaggtttttatattacagctccagatcctctacgccggacgcatcgtggccggcatcaccggcgccacaggtgcggttgctggcgcctatatcgccgacatcaccgatggggaagatcgggctcgccacttcgggctcatgagcgcttgtttcggcgtgggtatggtggcaggccccgtggccgggggactgttgggcgccatctccttgcatgcaccattccttgcggcggcggtgctcaacggcctcaacctactactgggctgcttcctaatgcaggagtcgcataagggagagcgtcgacatggatgagcgatgatgatatccgtttaggctgggcggtgatagcttctcgttcaggcagtacgcctcttttcttttccagacctgagggaggcggaaatggtgtgaggttcccggggaaaagccaaataggcgatcgcgggagtgctttatttgaagatcaggctatcactgcggtcaatagatttcacaatgtgatggctggacagcctgaggaactctcgaacccgaatggaaacaaccagatatttatgaatcagcgcggctcacatggcgttgtgctggcaaatgcaggttcatcctctgtctctatcaatacggcaacaaaattgcctgatggcaggtatgacaataaagctggagcgggttcatttcaagtgaacgatggtaaactgacaggcacgatcaatgccaggtctgtagctgtgctttatcctgatgatattgcaaaagcgcctcatgttttccttgagaattacaaaacaggtgtaacacattctttcaatgatcaactgacgattaccttgcgtgcagatgcgaatacaacaaaagccgtttatcaaatcaataatggaccagacgacaggcgtttaaggatggagatcaattcacaatcggaaaaggagatccaatttggcaaaacatacaccatcatgttaaaaggaacgaacagtgatggtgtaacgaggaccgagaaatacagttttgttaaaagagatccagcgtcggccaaaaccatcggctatcaaaatccgaatcattggagccaggtaaatgcttatatctataaacatgatgggagccgagtaattgaattgaccggatcttggcctggaaaaccaatgactaaaaatgcagacggaatttacacgctgacgctgcctgcggacacggatacaaccaacgcaaaagtgatttttaataatggcagcgcccaagtgcccggtcagaatcagcctggctttgattacgtgctaaatggtttatataatgactcgggcttaagcggttctcttccccattgatagcttggcgtaatcatggtcatagctgtttcctgtgtgaaattgttatccgctcacaattccacacaacatacgagccggaagcataaagtgtaaagcctggggtgcctaatgagtgagctaactcacattaattgcgttgcgctcactgcccgctttccagtcgggaaacctgtcgtgccagctgcattaatgaatcggccaacgcgcggggagaggcggtttgcgtattgggcgctcttccgcttcctcgctcactgactcgctgcgctcggtcgttcggctgcggcgagcggtatcagctcactcaaaggcggtaatacggttatccacagaatcaggggataacgcaggaaagaacatgtgagcaaaaggccagcaaaaggccaggaaccgtaaaaaggccgcgttgctggcgtttttccataggctccgcccccctgacgagcatcacaaaaatcgacgctcaagtcagaggtggcgaaacccgacaggactataaagataccaggcgtttccccctggaagctccctcgtgcgctctcctgttccgaccctgccgcttaccggatacctgtccgcctttctcccttcgggaagcgtggcgctttctcatagctcacgctgtaggtatctcagttcggtgtaggtcgttcgctccaagctgggctgtgtgcacgaaccccccgttcagcccgaccgctgcgccttatccggtaactatcgtcttgagtccaacccggtaagacacgacttatcgccactggcagcagccactggtaacaggattagcagagcgaggtatgtaggcggtgctacagagttcttgaagtggtggcctaactacggctacactagaagaacagtatttggtatctgcgctctgctgaagccagttaccttcggaaaaagagttggtagctcttgatccggcaaacaaaccaccgctggtagcggtggtttttttgtttgcaagcagcagattacgcgcagaaaaaaaggatctcaagaagatcctttgatcttttctacggggtctgacgctcagtggaacgaaaactcacgttaagggattttggtcatgagattatcaaaaaggatcttcacctagatccttttaaattaaaaatgaagttttaaatcaatctaaagtatatatgagtaaacttggtctgacagttaccaatgcttaatcagtgaggcacctatctcagcgatctgtctatttcgttcatccatagttgcctgactccccgtcgtgtagataactacgatacgggagggcttaccatctggccccagtgctgcaatgataccgcgagacccacgctcaccggctccagatttatcagcaataaaccagccagccggaagggccgagcgcagaagtggtcctgcaactttatccgcctccatccagtctattaattgttgccgggaagctagagtaagtagttcgccagttaatagtttgcgcaacgttgttgccattgctacaggcatcgtggtgtcacgctcgtcgtttggtatggcttcattcagctccggttcccaacgatcaaggcgagttacatgatcccccatgttgtgcaaaaaagcggttagctccttcggtcctccgatcgttgtcagaagtaagttggccgcagtgttatcactcatggttatggcagcactgcataattctcttactgtcatgccatccgtaagatgcttttctgtgactggtgagtactcaaccaagtcattctgagaatagtgtatgcggcgaccgagttgctcttgcccggcgtcaatacgggataataccgcgccacatagcagaactttaaaagtgctcatcattggaaaacgttcttcggggcgaaaactctcaaggatcttaccgctgttgagatccagttcgatgtaacccactcgtgcacccaactgatcttcagcatcttttactttcaccagcgtttctgggtgagcaaaaacaggaaggcaaaatgccgcaaaaaagggaataagggcgacacggaaatgttgaatactcatactcttcctttttcaatattattgaagcatttatcagggttattgtctcatgagcggatacatatttgaatgtatttagaaaaataaacaaataggggttccgcgcacatttccccgaaaagtgccacctgacgtctaagaaaccattattatcatgacattaacctataaaaataggcgtatcacgaggccctttcgtc